European Patent Application EP 4 461 741 A1, published November 13, 2024. Title: A MODIFIED YEAST STRAIN FOR LOW ALCOHOL FERMENTATION. Applicant: BRAIN Biotech AG. The sequence listing filed with the application follows.

SEQUENCE LISTING (18 sequences)

SEQ ID NO: 1 - protein, 240 aa, unidentified
MADEERLKEFKEANKIVFDPNTRQVWENQNRDGTKPATTFQSEEDMKRAAPESEKGTSATSGIVPTLQNIVATVTLGCRLDLKTVALHARNAEYNPKRFAAVIMRIREPKTTALIFAPGKMVVTGAKSEDDSKLASRKYARIIQKIGFAAKFTDFKIQNIVGSCDVKFPIRLEGLAFSHGTFSSYEPELFPGLIHRMVKPKIVLSIFVSGKIVLTGAKQREEIYQAFEAIYPVLSEFRKM

SEQ ID NO: 2 - DNA, 723 bp, unidentified
  source 1..723: mol_type = other DNA
atggccgatgaggaacgtttaaaggagtttaaagaggcaaacaagatagtgtttgatccaaataccagacaagtatgggaaaaccagaatcgagatggtacaaaaccagcaactactttccagagtgaagaggacatgaaaagagctgccccagaatctgaaaaaggtacctccgccacatcaggtattgttccaacactacaaaacattgtggcaactgtgactttggggtgcaggttagatctgaaaacagttgcgctacatgcccgtaatgcagaatataaccccaagcgttttgctgctgtcatcatgcgtattagagagccaaaaactacagctttaatttttgccccagggaaaatggttgttaccggtgcaaaaagtgaggatgactcaaagctggccagtagaaaatatgcaagaattatccaaaaaatcgggtttgctgctaaattcacagacttcaaaatacaaaatattgtcggttcgtgtgacgttaaattccctatacgtctagaagggttagcattcagtcatggtactttctcctcctatgagccagaattgtttcctggtttgatccatagaatggtgaagccgaaaattgtgttgagtatttttgtttcaggaaagattgttcttactggtgcaaagcaaagggaagaaatttaccaagcttttgaagctatataccctgtgctaagtgaatttagaaaaatgtga

SEQ ID NO: 3 - DNA, 3822 bp, unidentified
  source 1..3822: mol_type = other DNA
atgaagaacagcctggaagatttcaccaacctgtacagcctgcagaaaaccctgagattcgagctgaagcccatcggcaacacccagagcatgctggaagaggacggcgtgttcgacaccgacgagaagagaaagatcgcctacagcaagaccaagccttacatcgaccggctgcacagagagttcatcgaggaaagcctgagcgacgcccagatcagcaagctggacgagtacttcaaggcctacgtggactacaagaaggataagaaggacaccaagcggttcaaccggatcaagcagttcaagagcgtgctgcggaaagaagtggtggatcacttcaacaagcagggcaaagaatggaccaccgtgaagttcgcccacctgaagatcaagaaaaaggacctggaagtgctgttcgagaagcagctgcccaacatcctgaaagaggaatacggcaccgagaaagagacacagatcatcgacgaggacagcggcgaagtgaccagcatcttcgacatgtggaacggcttcatgggctacttcaccaagttcttcgagacacggaagaacttctacaagagcgacggcaccagcaccgccattgccaccagaatcatcgaccagaacctggacagattcatcgagaacatcctcatctacgacagcatcaagcccaagatcgacaccagcgaagtgcgcgagttcttcaacctggaaagcgacaccatcttcagcatggaattctacaacaactgcctgctgcaggccggcatcgatcagtacaacaatttcctcggcggcaagaccctggaaaacggcagaaagatccggggcatcaacgagctgatcaacaagtaccggcaagagaaccccgaggacaagatcccattcctgaagaagctggacaagcagatccacagcgagaaagaaaagttcatccagcagatcgagacactcgaggacctgaaagaagaactgcagaagttctacaactccagcaacgagaagattaagatcctggacaacctgctgtcccggatcgaggaattcaagcccgagggcatcttcatctccaagcaggccttcaacaccatcagcagacggtggaccgatcagagcgaggcctttgagacaagcctgttcgagtccctcaaagaggaaaagcccatcaccggcacagccaaaaagaaggatgacggctacaacttccccgagttcatctccctgcagagcatccggaacacactgaagaaggtgcagggcgaagagaggttctggaaagagcggtactaccgggacaacagcgagtctggaatcctggccggcaacgaggaaatctggacccagttcctgatgatcttcaagtccgagttcaacagcaagttcgagcggaacgaccctgaggacaatggcaccatcggctacaatctgtttaaagaggacctcgagaagctgctcaaggacctcaagatcaccaaggataccaagagcatcatcaagcgcttcgccgacgaggccctgcacatctatcaagtgggcaagtatttcgccctcgagaaagacagagtgtggatcagcagctacgacgacctgctggacaccttctacacagaccccaacaccggctacctgagcttttacgagggcgcctacgagcagatcgtgcagccctacaacatgatccggaactacctgaccagaaagccctactccgatgagaagtggaagctgaacttcgagaaccccacactggccaacggctgggacaagaacaaagagacagacaacagctccatcatgctgagaaaagaaggcgcctactacctgggcatcatgaagaagggcaagaacaagctgtttgaggaacggaaccggcagctgttcgaacccaagaacggcgaggatacctacgagaaactgagctataagctgttccccgatcctgccaagatgatccccaaagtgtgcttcagcaacaagaacatccagatgttcagccccagcaccgagatcatgaacatctacaacggcgagacattcaagaagaatagcgacgacttcagcgtgtcctccatgcagaagctgatcgccttttacaccaagtgcctgagccagtacgaaggctggaagtactacgacttcaagtacatcaagagccccgaccagtacaaggacaacatcggcgagttttacaacgacgtggccaagagcggctacagagtttggttcgagaatatcagccagagctacgtcgacagcaagaacaccatgggcgagctgtacctgttcaagatccacaacaaggactggaaccagaaggacaaaaagaccaaagtgggctccaagaacctgcacacccactacttcgaggaactgttcagccaggacaatattgagaacaactttccgctgaagctgaatggcgaggccgaggtgttctacagacccaagacaaacccagagaagctgggcaccaagaaggactctaagggcagagaagtgatcgaccggaagagatacgccagcgacaaggtgctgttccacgtgccaatcacactgaacagaacccctgtgaccaccaccaagctgaacaaagaaatcaacggcttcctggccaacaatcccagcatcaacatcatcggcgtggaccggggagagaagcacctggtgtactacagcgtggtcaaccagcggggcaaaatgctggaatccggctcctttaataccatcaacggcgtcgactaccacggcaaactggaagagagagccgatcggagagagcaggctagaagagactggcaggacgtggaaggcatcaagaatctgaagaaaggctacatcagcctggtcgtcagagagctggccaacctgagcatcaagtacaacgccatcatcgtgatggaagatctgaacatgcggtttaagcagatcagaggcggcatcgagaagtccgcctaccagcagctggaaaaggccctgatcgaaaagctgaattacctggtcaacaagaccgagacagaccctcagaaaaccggccacattctgaaggcctatcagctgacaagccccatcaagtcctttaaagagatgggcaagcagaccggcatcatcttctacacccaagccagctacaccagcgtgaccgatcctatcacaggctggcggcccaatctgtacctgaagtacagcagcgccagcaaggccaagtccgatatcctgaagttctccaagatctcctacaacaccaacaacaaccgcttcgagttcacctacgacctgcggaacttcgtgaacatgaaggcttatccccagaaaactgcctggaccatctgcagcaacgtggaaagattccgctgggacagaaagggcaacaaaaacaacggggagtacatccagtataaggacctgaccgagaatttcaagaccttctttgaggaagtgtccatcaactacaaaggcgacatcctgttccagatcaaaaacctgagcgagaaggggaacgagaagtttttccgggacctgatcttctatatcagcctgatctcccagatacggaacacccaaaaggacaagaagggcgacgagaacgacttcattctgagccccgtggaaccattcttcgacagcagaaagagcagcaccttcggcgagaatctgcccctgaacggggatgccaatggcgcctacaatatcgcccggaagggcatcattatgctgaacaagattagcaagggctccaaaaacaaagtcaaagaagatatcggctggggcgacctgtacatccctcacaccgagtgggatgatttcgccaccggctccatt

SEQ ID NO: 4 - DNA, 23 bp, unidentified
  source 1..23: mol_type = other DNA
gaactggaatatctttgtattcc

SEQ ID NO: 5 - DNA, 8235 bp, unidentified
  source 1..8235: mol_type = other DNA
agcttgcaaattaaagccttcgagcgtcccaaaaccttctcaagcaaggttttcagtataatgttacatgcgtacacgcgtctgtacagaaaaaaaagaaaaatttgaaatataaataacgttcttaatactaacataactataaaaaaataaatagggacctagacttcaggttgtctaactccttccttttcggttagagcggatgtggggggagggcgtgaatgtaagcgtgacataactaattacatgatatcgacaaaggaaaagggggacggatctccgaggcctcggacccgtcgggccgcgtcggacgtgtcagtcctgctcctcgcaattgttagaaaaactcatcgagcatcaaatgaaactgcaatttattcatatcaggattatcaataccatatttttgaaaaagccgtttctgtaatgaaggagaaaactcaccgaggcagttccataggatggcaagatcctggtatcggtctgcgattccgactcgtccaacatcaatacaacctattaatttcccctcgtcaaaaataaggttatcaagtgagaaatcaccatgagtgacgactgaatccggtgagaatggcaaaagcttatgcatttctttccagacttgttcaacaggccagccattacgctcgtcatcaaaatcactcgcatcaaccaaaccgttattcattcgtgattgcgcctgagcgaggcgaaatacgcgatcgctgttaaaaggacaattacaaacaggaatcgaatgcaaccggcgcaggaacactgccagcgcatcaacaatattttcacctgaatcaggatattcttctaatacctggaatgctgttttgccggggatcgcagtggtgagtaaccatgcatcatcaggagtacggataaaatgcttgatggtcggaagaggcataaattccgtcagccagtttagtctgaccatctcatctgtaacatcattggcaacgctacctttgccatgtttcagaaacaactctggcgcatcgggcttcccatacaatcgatagattgtcgcacctgattgcccgacattatcgcgagcccatttatacccatataaatcagcatccatgttggaatttaatcgcggcctcgaaacgtgagtcttttccttacccatggtttagttcctcaccttgtcgtattatactatgccgatatactatgccgatgattaattgtcaacaccgcccttagattagattgctatgctttctttctaatgagcaagaagtaaaaaaagttgtaatagaacaagaaaaatgaaactgaaacttgagaaattgaagaccgtttattaacttaaatatcaatgggaggtcatcgaaagagaaaaaaatcaaaaaaaaaaattttcaagaaaaagaaacgtgataaaaatttttattgcctttttcgacgaagaaaaagaaacgaggcggtctcttttttcttttccaaacctttagtacgggtaattaacgacaccctagaggaagaaagaggggaaatttagtatgctgtgcttgggtgttttgaagtggtacggcgatgcgcggagtccgagaaaatctggaagagtaaaaaaggagtagaaacattttgaagctatggtgtgtgggggatccgcacaaacgaaggtctcactgatcgcttgcctgtaacttacacgcgcctcgtatcttttaatgatggaataatttgggaatttactctgtgtttatttatttttatgttttgtatttggattttagaaagtaaataaagaaggtagaagagttacggaatgaagaaaaaaaaataaacaaaggtttaaaaaatttcaacaaaaagcgtactttacatatatatttattagacaagaaaagcagattaaatagatatacattcgattaacgataagtaaaatgtaaaatcacaggattttcgtgtgtggtcttctacacagacaagatgaaacaattcggcattaatacctgagagcaggaagagcaagataaaaggtagtatttgttggcgatccccctagagtcttttacatcttcggaaaacaaaaactattttttctttaatttctttttttactttctatttttaatttatatatttatattaaaaaatttaaattataattatttttatagcacgtgatgaaaaggacccatcgataagctggtacgcgccatatggcctgcaggtttaaagattacggatatttaacttacttagaataatgccatttttttgagttataataatcctacgttagtgtgagcgggatttaaactgtgaggaccttaatacattcagacacttctgcggtatcaccctacttattcccttcgagattatatctaggaacccatcaggttggtggaagattacccgttctaagacttttcagcttcctctattgatgttacacctggacaccccttttctggcatccagtttttaatcttcagtggcatgtgagattctccgaaattaattaaagcaatcacacaatgctctcggataccacctcggttgaaactgacaggtggtttgttacgcatgctaatgcaaaggagcctatatacctttggctcggctgctgtaacagggaatataaagggcagcataatttaggagtttagtgaacttgcaacatttactattttcccttcttacgtaaatatttttctttttaattctaaatcaatctttttcaattttttgtttgtattcttttcttgcttaaatctataactacaaaaaacacatacataaactaaaaatggccgactacaaggacgacgacgataagggcgctgccgagaacctgtactttcagtctcctgccgccaagaagaagaaactggacggcagcgtggacatgaagaacagcctggaagatttcaccaacctgtacagcctgcagaaaaccctgagattcgagctgaagcccatcggcaacacccagagcatgctggaagaggacggcgtgttcgacaccgacgagaagagaaagatcgcctacagcaagaccaagccttacatcgaccggctgcacagagagttcatcgaggaaagcctgagcgacgcccagatcagcaagctggacgagtacttcaaggcctacgtggactacaagaaggataagaaggacaccaagcggttcaaccggatcaagcagttcaagagcgtgctgcggaaagaagtggtggatcacttcaacaagcagggcaaagaatggaccaccgtgaagttcgcccacctgaagatcaagaaaaaggacctggaagtgctgttcgagaagcagctgcccaacatcctgaaagaggaatacggcaccgagaaagagacacagatcatcgacgaggacagcggcgaagtgaccagcatcttcgacatgtggaacggcttcatgggctacttcaccaagttcttcgagacacggaagaacttctacaagagcgacggcaccagcaccgccattgccaccagaatcatcgaccagaacctggacagattcatcgagaacatcctcatctacgacagcatcaagcccaagatcgacaccagcgaagtgcgcgagttcttcaacctggaaagcgacaccatcttcagcatggaattctacaacaactgcctgctgcaggccggcatcgatcagtacaacaatttcctcggcggcaagaccctggaaaacggcagaaagatccggggcatcaacgagctgatcaacaagtaccggcaagagaaccccgaggacaagatcccattcctgaagaagctggacaagcagatccacagcgagaaagaaaagttcatccagcagatcgagacactcgaggacctgaaagaagaactgcagaagttctacaactccagcaacgagaagattaagatcctggacaacctgctgtcccggatcgaggaattcaagcccgagggcatcttcatctccaagcaggccttcaacaccatcagcagacggtggaccgatcagagcgaggcctttgagacaagcctgttcgagtccctcaaagaggaaaagcccatcaccggcacagccaaaaagaaggatgacggctacaacttccccgagttcatctccctgcagagcatccggaacacactgaagaaggtgcagggcgaagagaggttctggaaagagcggtactaccgggacaacagcgagtctggaatcctggccggcaacgaggaaatctggacccagttcctgatgatcttcaagtccgagttcaacagcaagttcgagcggaacgaccctgaggacaatggcaccatcggctacaatctgtttaaagaggacctcgagaagctgctcaaggacctcaagatcaccaaggataccaagagcatcatcaagcgcttcgccgacgaggccctgcacatctatcaagtgggcaagtatttcgccctcgagaaagacagagtgtggatcagcagctacgacgacctgctggacaccttctacacagaccccaacaccggctacctgagcttttacgagggcgcctacgagcagatcgtgcagccctacaacatgatccggaactacctgaccagaaagccctactccgatgagaagtggaagctgaacttcgagaaccccacactggccaacggctgggacaagaacaaagagacagacaacagctccatcatgctgagaaaagaaggcgcctactacctgggcatcatgaagaagggcaagaacaagctgtttgaggaacggaaccggcagctgttcgaacccaagaacggcgaggatacctacgagaaactgagctataagctgttccccgatcctgccaagatgatccccaaagtgtgcttcagcaacaagaacatccagatgttcagccccagcaccgagatcatgaacatctacaacggcgagacattcaagaagaatagcgacgacttcagcgtgtcctccatgcagaagctgatcgccttttacaccaagtgcctgagccagtacgaaggctggaagtactacgacttcaagtacatcaagagccccgaccagtacaaggacaacatcggcgagttttacaacgacgtggccaagagcggctacagagtttggttcgagaatatcagccagagctacgtcgacagcaagaacaccatgggcgagctgtacctgttcaagatccacaacaaggactggaaccagaaggacaaaaagaccaaagtgggctccaagaacctgcacacccactacttcgaggaactgttcagccaggacaatattgagaacaactttccgctgaagctgaatggcgaggccgaggtgttctacagacccaagacaaacccagagaagctgggcaccaagaaggactctaagggcagagaagtgatcgaccggaagagatacgccagcgacaaggtgctgttccacgtgccaatcacactgaacagaacccctgtgaccaccaccaagctgaacaaagaaatcaacggcttcctggccaacaatcccagcatcaacatcatcggcgtggaccggggagagaagcacctggtgtactacagcgtggtcaaccagcggggcaaaatgctggaatccggctcctttaataccatcaacggcgtcgactaccacggcaaactggaagagagagccgatcggagagagcaggctagaagagactggcaggacgtggaaggcatcaagaatctgaagaaaggctacatcagcctggtcgtcagagagctggccaacctgagcatcaagtacaacgccatcatcgtgatggaagatctgaacatgcggtttaagcagatcagaggcggcatcgagaagtccgcctaccagcagctggaaaaggccctgatcgaaaagctgaattacctggtcaacaagaccgagacagaccctcagaaaaccggccacattctgaaggcctatcagctgacaagccccatcaagtcctttaaagagatgggcaagcagaccggcatcatcttctacacccaagccagctacaccagcgtgaccgatcctatcacaggctggcggcccaatctgtacctgaagtacagcagcgccagcaaggccaagtccgatatcctgaagttctccaagatctcctacaacaccaacaacaaccgcttcgagttcacctacgacctgcggaacttcgtgaacatgaaggcttatccccagaaaactgcctggaccatctgcagcaacgtggaaagattccgctgggacagaaagggcaacaaaaacaacggggagtacatccagtataaggacctgaccgagaatttcaagaccttctttgaggaagtgtccatcaactacaaaggcgacatcctgttccagatcaaaaacctgagcgagaaggggaacgagaagtttttccgggacctgatcttctatatcagcctgatctcccagatacggaacacccaaaaggacaagaagggcgacgagaacgacttcattctgagccccgtggaaccattcttcgacagcagaaagagcagcaccttcggcgagaatctgcccctgaacggggatgccaatggcgcctacaatatcgcccggaagggcatcattatgctgaacaagattagcaagggctccaaaaacaaagtcaaagaagatatcggctggggcgacctgtacatccctcacaccgagtgggatgatttcgccaccggctccattaagaggccagccgccacaaagaaagccggacaggctaaaaagaagaaggccagcggaagcggcgctggcagcccgaaaaagaaacgcaaggtggaagatcccaagaagaaacggaaagtctgagcggccgcaatgccggcgcaatgattgaatagtcaaagattttttttttttaattttttttttttaattttttttttttttcatagaactttttatttaaataaatcacgtctatatatgtatcagtataacgtaaaaaaaaaaacaccgtcagttaaacaaaacataaataaaaaaaaaaagaagtgtcaaatcaagtgtcaaatggccctgcattaatgaatcggccaacgcgcggggagaggcggtttgcgtattgggcgctcttccgcttcctcgctcactgactcgctgcgctcggtcgttcggctgcggcgagcggtatcagctcactcaaaggcggtaatacggttatccacagaatcaggggataacgcaggaaagaacatgtgagcaaaaggccagcaaaaggccaggaaccgtaaaaaggccgcgttgctggcgtttttccataggctccgcccccctgacgagcatcacaaaaatcgacgctcaagtcagaggtggcgaaacccgacaggactataaagataccaggcgtttccccctggaagctccctcgtgcgctctcctgttccgaccctgccgcttaccggatacctgtccgcctttctcccttcgggaagcgtggcgctttctcatagctcacgctgtaggtatctcagttcggtgtaggtcgttcgctccaagctgggctgtgtgcacgaaccccccgttcagcccgaccgctgcgccttatccggtaactatcgtcttgagtccaacccggtaagacacgacttatcgccactggcagcagccactggtaacaggattagcagagcgaggtatgtaggcggtgctacagagttcttgaagtggtggcctaactacggctacactagaagaacagtatttggtatctgcgctctgctgaagccagttaccttcggaaaaagagttggtagctcttgatccggcaaacaaaccaccgctggtagcggtggtttttttgtttgcaagcagcagattacgcgcagaaaaaaaggatctcaagaagatcctttgatcttttctacggggtctgacgctcagtggaacgaaaactcacgttaagggattttggtcatgagattatcaaaaaggatcttcacctagatccttttaaattaaaaatgaagttttaaatcaatctaaagtatatatgagtaaacttggtctgacagttaccaatgcttaatcagtgaggcacctatctcagcgatctgtctatttcgttcatccatagttgcctgactccccgtcgtgtagataactacgatacgggagggcttaccatctggccccagtgctgcaatgataccgcgagacccacgctcaccggctccagatttatcagcaataaaccagccagccggaagggc

SEQ ID NO: 6 - DNA, 6488 bp, unidentified
  source 1..6488: mol_type = other DNA
ccccgtagaaaagatcaaaggatcttcttgagatcctttttttctgcgcgtaatctgctgcttgcaaacaaaaaaaccaccgctaccagcggtggtttgtttgccggatcaagagctaccaactctttttccgaaggtaactggcttcagcagagcgcagataccaaatactgtccttctagtgtagccgtagttaggccaccacttcaagaactctgtagcaccgcctacatacctcgctctgctaatcctgttaccagtggctgctgccagtggcgataagtcgtgtcttaccgggttggactcaagacgatagttaccggataaggcgcagcggtcgggctgaacggggggttcgtgcacacagcccagcttggagcgaacgacctacaccgaactgagatacctacagcgtgagctatgagaaagcgccacgcttcccgaagggagaaaggcggacaggtatccggtaagcggcagggtcggaacaggagagcgcacgagggagcttccagggggaaacgcctggtatctttatagtcctgtcgggtttcgccacctctgacttgagcgtcgatttttgtgatgctcgtcaggggggcggagcctatggaaaaacgccagcaacgcggcctttttacggttcctgggcttttgctggccttttgctcacatgttctttcctgcgttatcccctgattctgtggataaccgtattaccgcctttgagtgagctgataccgctcgccgcagccgaacgaccgagcgcagcgagtcagtgagcgaggaagcggaagagcgcccaatacgcaaaccgcctctccccgcgcgttggccgattcattaatgcagggccgcagcttgcaaattaaagccttcgagcgtcccaaaaccttctcaagcaaggttttcagtataatgttacatgcgtacacgcgtctgtacagaaaaaaaagaaaaatttgaaatataaataacgttcttaatactaacataactataaaaaaataaatagggacctagacttcaggttgtctaactccttccttttcggttagagcggatgtggggggagggcgtgaatgtaagcgtgacataactaattacatgatgcggccctctagatgcatgctcgaggagctcggatcccggtctgcatctgcggatcctctttgaaaagataatgtatgattatgctttcactcatatttatacagaaacttgatgttttctttcgagtatatacaaggtgattacatgtacgtttgaagtacaactctagattttgtagtgccctcttgggctagcggtaaaggtgcgcattttttcacaccctacaatgttctgttcaaaagattttggtcaaacgctgtagaagtgaaagttggtgcgcatgtttcggcgttcgaaacttctccgcagtgaaagataaatgatctagttttcacaagaaaacaagcgcaagtggtttagtggtaaaatccaacgttgccatcgttgggcccccggttcgattccgggcttgcgcaaatttctactgttgtagatgaactggaatatctttgtattccatttattttttgtcactattgttatgtaaaatgccacctctgacagtatggaacgcaaacttctgtctagtggataacagaatttttctatggccaatttaaccggtgaggacgaggacgcacggaggagagtcttccttcggagggctgtcacccgctcggcggcttctaatccgtggactagtggatcgatccccacgcgccctgtagcggcgcattaagcgcggcgggtgtggtggttacgcgcagcgtgaccgctacacttcccaccgccctagcccccgctcctttcgctttcttcccttcctttctcgccacgttcgccggctttccccgtcaagctctaaatgggggcatccgtttacccttccgatttactgctttacggcacctcgaccccaaaaaacttgattagggtgatggttcacgtagtgggccatcgccctgatagaccctttttcgccctttgacgttggagtccacgttctttaatagtggactcttgttggaaactggaacaacactcaaccctatctcggtctattcttttgatttataagggattttgccgatttcgggctattcgttaaaaaatgagctgatttaacaaaaatttaacgcgaattttaacaaaatattaacgtttacaatttaaatatttgcttatacaatcttcctgtttttggggcttttctgattatcaaccggggtggagcttcccattgcgaataccgcttccacaaacattgctcaaaagtatctctttgctatatatctctgtgctatatccctatataacctacccatccacctttcgctccttgaacttgcatctaaactcgacctctacattttttatgtttatctctagtattactctttagacaaaaaaattgtagtaagaactattcatagagtgaatcgaaaacaatacgaaaatgtaaacatttcctatacgtagtatatagagacaaaatagaagaaaccgttcataattttctgaccaatgaagaatcatcaacgctatcactttctgttcacaaagtatgcgcaatccacatcggtatagaatataatcggggatgcctttatcttgaaaaaatgcacccgcagcttcgctagtaatcagtaaacgcgggaagtggagtcaggctttttttatggaagagaaaatagacaccaaagtagccttcttctaaccttaacggacctacagtgcaaaaagttatcaagagactgcattatagagcgcacaaaggagaaaaaaagtaatctaagatgctttgttagaaaaatagcgctctcgggatgcatttttgtagaacaaaaaagaagtatagattctttgttggtaaaatagcgctctcgcgttgcatttctgttctgtaaaaatgcagctcagattctttgtttgaaaaattagcgctctcgtcgcgttgcatttttgttttacaaaaatgaagcacagattcttcgttggtaaaatagcgctttcgcgttgcatttctgttctgtaaaaatgcagctcagattctttgtttgaaaaattagcgctctcgcgttgcatttttgttctacaaaatgaagcacagatgcttcgttaacaaagatatgctattgaagtgcaagatggaaacgcagaaaatgaaccggggatgcgacgtgcaagattacctatgcaatagatgcaatagtttctccaggaaccgaaatacatacattgtcttccgtaaagcgctagactatatattattatacaggttcaaatatactatctgtttcagggaaaactcccaggttcggatgttcaaaattcaatgatgggtaacaagtacgatcgtaaatctgtaaaacagtttgtcggatattaggctgtatctcctcaaagcgtattcgaatatcattgagaagctgcagcgtcacatcggataataatgatggcagccattgtagaagtgccttttgcatttctagtctctttctcggtctagctagttttactacatcgcgaagatagaatcttagatcacactgcctttgctgagctggatcaatagagtaacaaaagagtggtaaggcctcgttaaaggacaaggacctgagcggaagtgtatcgtacagtagacggagtatctagtatagtctatagtccgtggaattaattctcatctttgacagcttatcatcgataagtttagcttgcctcgtccccgccgggtcacccggccagcgacatggaggcccagaataccctccttgacagtcttgacgtgcgcagctcaggggcatgatgtgactgtcgcccgtacatttagcccatacatccccatgtataatcatttgcatccatacattttgatggccgcacggcgcgaagcaaaaattacggctcctcgctgcagacctgcgagcagggaaacgctcccctcacagacgcgttgaattgtccccacgccgcgcccctgtagagaaatataaaaggttaggatttgccactgaggttcttctttcatatacttccttttaaatcttgctaggatacagttctcacatcacatccgaacataaacaaccatgggtaaaaagcctgaactcaccgcgacgtctgtcgagaagtttctgatcgaaaagttcgacagcgtctccgacctgatgcagctctcggagggcgaagaatctcgtgctttcagcttcgatgtaggagggcgtggatatgtcctgcgggtaaatagctgcgccgatggtttctacaaagatcgttatgtttatcggcactttgcatcggccgcgctcccgattccggaagtgcttgacattggggaatttagcgagagcctgacctattgcatctcccgccgtgcacagggtgtcacgttgcaagacctgcctgaaaccgaactgcccgctgttctgcagccggtcgcggaggcaatggatgcgatcgctgcggccgatcttagccagacgagcgggttcggcccattcggaccgcaaggaatcggtcaatacactacatggcgtgatttcatatgcgcgattgctgatccccatgtgtatcactggcaaactgtgatggacgacaccgtcagtgcgtccgtcgcgcaggctctcgatgagctgatgctttgggccgaggactgccccgaagtccggcacctcgtgcacgcggatttcggctccaacaatgtcctgacggacaatggccgcataacagcggtcattgactggagcgaggcgatgttcggggattcccaatacgaggtcgccaacatcttcttctggaggccgtggttggcttgtatggagcagcagacgcgctacttcgagcggaggcatccggagcttgcaggatcgccgcggctccgggcgtatatgctccgcattggtcttgaccaactctatcagagcttggttgacggcaatttcgatgatgcagcttgggcgcagggtcgatgcgacgcaatcgtccgatccggagccgggactgtcgggcgtacacaaatcgcccgcagaagcgcggccgtctggaccgatggctgtgtagaagtactcgccgatagtggaaaccgacgccccagcactcgtccgagggcaaaggaataatcagtactgacaataaaaagattcttgttttcaagaacttgtcatttgtatagtttttttatattgtagttgttctattttaatcaaatgttagcgtgatttatattttttttcgcctcgacatcatctgcccagatgcgaagttaagtgcgcagaaagtaatatcatgcgtcaatcgtatgtgaatgctggtcgctatactgctgtcgattcgatactaacgccgccatccagtgtcgaaaatactaaactcacaaattagagcttcaatttaattatatcagttattacccattgaaaaaggaagagtatgagtattcaacatttccgtgtcgcccttattcccttttttgcggcattttgccttcctgtttttgctcacccagaaacgctggtgaaagtaaaagatgctgaagatcagttgggtgcacgagtgggttacatcgaactggatctcaacagcggtaagatccttgagagttttcgccccgaagaacgttttccaatgatgagcacttttaaagttctgctatgtgatacactattatcccgtattgacgccgggcaagagcaactcggtcgccgcatacactattctcagaatgacttggttgagtactcaccagtcacagaaaagcatcttacggatggcatgacagtaagagaattatgcagtgctgccataaccatgagtgataacactgcggccaacttacttctgacaacgatcggaggaccgaaggagctaaccgcttttttgcacaacatgggggatcatgtaactcgccttgatcgttgggaaccggagctgaatgaagccataccaaacgacgagagtgacaccacgatgcctgtagcaatgccaacaacgttgcgcaaactattaactggcgaactacttactctagcttcccggcaacaattaatagactgaatggaggcggataaagttgcaggaccacttctgcgctcggcccttccggctggctggtttattgctgataaatctggagccggtgagcgtgggtctcgcggtatcattgcagcactggggccagatggtaagcgctcccgtatcgtagttatctacacgacggggagtcaggcaactatggatgaacgaaatagacagatcgctgagataggtgcctcactgattaagcattggtaactgtcagaccaagtttactcatatatactttagattgatttaaaacttcatttttaatttaaaaggatctaggtgaagatcctttttgataatctcatgaccaaaatcccttaacgtgagttttcgttccactgagcgtcaga

SEQ ID NO: 7 - DNA, 1760 bp, unidentified
  source 1..1760: mol_type = other DNA
gttgttgtctcaccatatccgcaatgacaaaaaaatgatggaagacactaaaggaaaaaattaacgacaaagacagcaccaacagatgtcgttgttccagagctgatgaggggtatctcgaagcacacgaaactttttccttccttcattcacgcacactactctctaatgagcaacggtatacggccttccttccagttacttgaatttgaaataaaaaaagtttgctgtcttgctatcaagtataaatagaactgcaattattaatcttttgttttctcgtcattgttctcgttccctttcttccttgtttctttttctgcacaatatttcaagctataccaagcatacaatcaactatctcatatacaatggccgatgaggaacgtttaaaggagtttaaagaggcaaacaagatagtgtttgatccaaataccagacaagtatgggaaaaccagaatcgagatggtacaaaaccagcaactactttccagagtgaagaggacatgaaaagagctgccccagaatctgaaaaaggtacctccgccacatcaggtattgttccaacactacaaaacattgtggcaactgtgactttggggtgcaggttagatctgaaaacagttgcgctacatgcccgtaatgcagaatataaccccaagcgttttgctgctgtcatcatgcgtattagagagccaaaaactacagctttaatttttgccccagggaaaatggttgttaccggtgcaaaaagtgaggatgactcaaagctggccagtagaaaatatgcaagaattatccaaaaaatcgggtttgctgctaaattcacagacttcaaaatacaaaatattgtcggttcgtgtgacgttaaattccctatacgtctagaagggttagcattcagtcatggtactttctcctcctatgagccagaattgtttcctggtttgatccatagaatggtgaagccgaaaattgtgttgagtatttttgtttcaggaaagattgttcttactggtgcaaagcaaagggaagaaatttaccaagcttttgaagctatataccctgtgctaagtgaatttagaaaaatgtgatggggaaggagtagacgaaaagaaaaaaaggttttctatttgttccattttctcaattattaatggtcctcaaagaaataaaagaaaaggaagaagaagtaattgtaatatcaaacggttttttatagtatattcttcttattctatatttatatatcaatgttttataataagatgtttattcatagcatatctggtggatcgtctctattaagcgccagcgaggtgtttgcctctgcatttttcagcaaagcaagctccctttccagcttgaatctatgttcacgctcatccgacaacgaatttcttatgatttatgatttttattattaaataagttataaaaaaataagtgtatacaaattttaaagtgactcttaggttttaaaacgaaaattcttattcttgagtaactctttcctgtaggtcaggttgctttctcaggtatagcatgaggtcgctcttattgaccacatctctaccggcatgccgagcaaatgcctgcaaatcgctccccatttcacccaattgtagatatgctaactccagcaatgagttgatgaatctcggtgtgtattttatgtcctcagaggacaacacctgttgtaatcgttcttccacacggatccacagcctagccttcagttgggctctatcttcatcgtc

SEQ ID NO: 8 - DNA, 723 bp, Saccharomyces cerevisiae
  source 1..723: mol_type = other DNA
atggccgatgaggaacgtttaaaggagtttaaagaggcaaacaagatagtgtttgatccaaataccagacaagtatgggaaaaccagaatcgagatggtacaaaaccagcaactactttccagagtgaagaggacataaaaagagctgccccagaatctgaaaaagacacctccgccacatcaggtattgttccaacactacaaaacattgtggcaactgtgactttggggtgcaggttagatctgaaaacagttgcgctacatgcccgtaatgcagaatataaccccaagcgttttgctgctgtcatcatgcgtattagagagccaaaaactacagctttaatttttgcctcagggaaaatggttgttaccggtgcaaaaagtgaggatgactcaaagctggccagtagaaaatatgcaagaattatccaaaaaatcgggtttgctgctaaattcacagacttcaaaatacaaaatattgtcggttcgtgtgacgttaaattccctatacgtctagaagggttagcattcagtcatggtactttctcctcctatgagccagaattgtttcctggtttgatctatagaatggtgaagccgaaaattgtgttgttaatttttgtttcaggaaagattgttcttactggtgcaaagcaaagggaagaaatttaccaagcttttgaagctatataccctgtgctaagtgaatttagaaaaatgtga

SEQ ID NO: 9 - protein, 240 aa, Saccharomyces cerevisiae
MADEERLKEFKEANKIVFDPNTRQVWENQNRDGTKPATTFQSEEDIKRAAPESEKDTSATSGIVPTLQNIVATVTLGCRLDLKTVALHARNAEYNPKRFAAVIMRIREPKTTALIFASGKMVVTGAKSEDDSKLASRKYARIIQKIGFAAKFTDFKIQNIVGSCDVKFPIRLEGLAFSHGTFSSYEPELFPGLIYRMVKPKIVLLIFVSGKIVLTGAKQREEIYQAFEAIYPVLSEFRKM

SEQ ID NO: 10 - protein, 348 aa, Saccharomyces cerevisiae
MSIPETQKGVIFYESHGKLEYKDIPVPKPKANELLINVKYSGVCHTDLHAWHGDWPLPVKLPLVGGHEGAGVVVGMGENVKGWKIGDYAGIKWLNGSCMACEYCELGNESNCPHADLSGYTHDGSFQQYATADAVQAAHIPQGTDLAQVAPILCAGITVYKALKSANLMAGHWVAISGAAGGLGSLAVQYAKAMGYRVLGIDGGEGKEELFRSIGGEVFIDFTKEKDIVGAVLKATDGGAHGVINVSVSEAAIEASTRYVRANGTTVLVGMPAGAKCCSDVFNQVVKSISIVGSYVGNRADTREALDFFARGLVKSPIKVVGLSTLPEIYEKMEKGQIVGRYVVDTSK

SEQ ID NO: 11 - protein, 348 aa, Saccharomyces cerevisiae
MSIPETQKAIIFYESNGKLEHKDIPVPKPKPNELLINVKYSGVCHTDLHAWHGDWPLPTKLPLVGGHEGAGVVVGMGENVKGWKIGDYAGIKWLNGSCMACEYCELGNESNCPHADLSGYTHDGSFQEYATADAVQAAHIPQGTDLAEVAPILCAGITVYKALKSANLRAGHWAAISGAAGGLGSLAVQYAKAMGYRVLGIDGGPGKEELFTSLGGEVFIDFTKEKDIVSAVVKATNGGAHGIINVSVSEAAIEASTRYCRANGTVVLVGLPAGAKCSSDVFNHVVKSISIVGSYVGNRADTREALDFFARGLVKSPIKVVGLSSLPEIYEKMEKGQIAGRYVVDTSK

SEQ ID NO: 12 - protein, 375 aa, Saccharomyces cerevisiae [sequence omitted]

SEQ ID NO: 13 - protein, 382 aa, Saccharomyces cerevisiae
MSSVTGFYIPPISFFGEGALEETADYIKNKDYKKALIVTDPGIAAIGLSGRVQKMLEERDLNVAIYDKTQPNPNIANVTAGLKVLKEQNSEIVVSIGGGSAHDNAKAIALLATNGGEIGDYEGVNQSKKAALPLFAINTTAGTASEMTRFTIISNEEKKIKMAIIDNNVTPAVAVNDPSTMFGLPPALTAATGLDALTHCIEAYVSTASNPITDACALKGIDLINESLVAAYKDGKDKKARTDMCYAEYLAGMAFNNASLGYVHALAHQLGGFYHLPHGVCNAVLLPHVQEANMQCPKAKKRLGEIALHFGASQEDPEETIKALHVLNRTMNIPRNLKELGVKTEDFEILAEHAMHDACHLTNPVQFTKEQVVAIIKKAYEY

SEQ ID NO: 14 - protein, 351 aa, Saccharomyces cerevisiae
MPSQVIPEKQKAIVFYETDGKLEYKDVTVPEPKPNEILVHVKYSGVCHSDLHAWHGDWPFQLKFPLIGGHEGAGVVVKLGSNVKGWKVGDFAGIKWLNGTCMSCEYCEVGNESQCPYLDGTGFTHDGTFQEYATADAVQAAHIPPNVNLAEVAPILCAGITVYKALKRANVIPGQWVTISGACGGLGSLAIQYALAMGYRVIGIDGGNAKRKLFEQLGGEIFIDFTEEKDIVGAIIKATNGGSHGVINVSVSEAAIEASTRYCRPNGTVVLVGMPAHAYCNSDVFNQVVKSISIVGSCVGNRADTREALDFFARGLIKSPIHLAGLSDVPEIFAKMEKGEIVGRYVVETSK

SEQ ID NO: 15 - protein, 386 aa, Saccharomyces cerevisiae
MSAATVGKPIKCIAAVAYDAKKPLSVEEITVDAPKAHEVRIKIEYTAVCHTDAYTLSGSDPEGLFPCVLGHEGAGIVESVGDDVITVKPGDHVIALYTAECGKCKFCTSGKTNLCGAVRATQGKGVMPDGTTRFHNAKGEDIYHFMGCSTFSEYTVVADVSVVAIDPKAPLDAACLLGCGVTTGFGAALKTANVQKGDTVAVFGCGTVGLSVIQGAKLRGASKIIAIDINNKKKQYCSQFGATDFVNPKEDLAKDQTIVEKLIEMTDGGLDFTFDCTGNTKIMRDALEACHKGWGQSIIIGVAAAGEEISTRPFQLVTGRVWKGSAFGGIKGRSEMGGLIKDYQKGALKVEEFITHRRPFKEINQAFEDLHNGDCLRTVLKSDEIK

SEQ ID NO: 16 - protein, 500 aa, Saccharomyces cerevisiae
MTKLHFDTAEPVKITLPNGLTYEQPTGLFINNKFMKAQDGKTYPVEDPSTENTVCEVSSATTEDVEYAIECADRAFHDTEWATQDPRERGRLLSKLADELESQIDLVSSIEALDNGKTLALARGDVTIAINCLRDAAAYADKVNGRTINTGDGYMNFTTLEPIGVCGQIIPWNFPIMMLAWKIAPALAMGNVCILKPAAVTPLNALYFASLCKKVGIPAGVVNIVPGPGRTVGAALTNDPRIRKLAFTGSTEVGKSVAVDSSESNLKKITLELGGKSAHLVFDDANIKKTLPNLVNGIFKNAGQICSSGSRIYVQEGIYDELLAAFKAYLETEIKVGNPFDKANFQGAITNRQQFDTIMNYIDIGKKEGAKILTGGEKVGDKGYFIRPTVFYDVNEDMRIVKEEIFGPVVTVAKFKTLEEGVEMANSSEFGLGSGIETESLSTGLKVAKMLKAGTVWINTYNDFDSRVPFGGVKQSGYGREMGEEVYHAYTEVKAVRIKL

SEQ ID NO: 17 - protein, 925 aa, Saccharomyces cerevisiae
MLSIQQRYNICLMAERHPKWTQLELAKWAYETFQLPKIPSQGTISRLLARKSTYMNCKEHEKDANRLRKPNNLLVRKILQEWISQSLWNGIPITSPIIQDTAQAVWHRIPAEHREGNGSFSYKWISNFLSKMDVNISVLDEELPKTPKVWTFEERDVLKAYFSKIPPKDLFTLDEAFLSYNLPLDYAQYEASSIQRRIEVATVMLCSNLDGSEKLKPVVVGKYDSYKSFRNYFPNEPNDPVSQSMLGTKMAKKFDISYHSNRKAWLTSNLFHNWLVRWDKRLVAVNRKIWIVLDDSCCHRIINLRLQNIKLVYTSSNSKFLPFNWGVWDEFKTRYRIQQYQALIDLQNRISKNIQNKNKSERNECIPNGKKCLISFEQSQLTMSNAFKFIKKAWDDIPVDAIKANWKSSGLLPPEMIHLNENVSMAFKKNEVLESVLNRLCDEYYCVKKWEYEMLLDLNIENKNTNFLSTEELVESAIVEPCEPDFDTAPKGNEVHDDNFDVSVFANEDDNNQNHLSMSQASHNPDYNSNHSNNAIENTNNRGSNNNNNNNGSSNNINDNDSSVKYLQQNTVDNSTKTGNPGQPNISSMESQRNSSTTDLVVDGNYDVNFNGLLNDPYNTMKQPGPLDYNVSTLIDKPNLFLSPDLDLSTVGVDMQLPSSEYFSEVFSSAIRNNEKAASDQNKSTDELPSSTAMANSNSITTALLESRNQAQPFDVPHMNGLLSDTSKSGHSVNSSNAISQNSLNNFQHNSASVAEASSPSITPSPVAINSTGAPARSIISAPIDSNSSASSPSALEHLEGAVSGMSPSSTTILSNLQTNINIAKSLSTIMKHAESNEISLTKETINELNFNYLTLLKRIKKTRKQLNSESIKINSKNAQDHLETLLSGAAAAAATSANNLDLPTGGSNLPDSNNLHLPGNTGFF

SEQ ID NO: 18 - protein, 248 aa, Saccharomyces cerevisiae
MARTFFVGGNFKLNGSKQSIKEIVERLNTASIPENVEVVICPPATYLDYSVSLVKKPQVTVGAQNAYLKASGAFTGENSVDQIKDVGAKWVILGHSERRSYFHEDDKFIADKTKFALGQGVGVILCIGETLEEKKAGKTLDVVERQLNAVLEEVKDWTNVVVAYEPVWAIGTGLAATPEDAQDIHASIRKFLASKLGDKAASELRILYGGSANGSNAVTFKDKADVDGFLVGGASLKPEFVDIINSRN